European Patent Application EP 4 512 897 A1, published February 26, 2025. Title: MUTANT OF SMALL MOLECULE CHAPERONE PROTEIN MOG1-ENCODING GENE AND USE THEREOF. Applicant: HUAZHONG UNIVERSITY OF SCIENCE AND TECHNOLOGY. The sequence listing filed with the application follows.

SEQUENCE LISTING (2 sequences)

SEQ ID NO: 1 - DNA, 847 bp, Artificial Sequence
  MOG1 gene mutant
ggagctaagccagacccgggtggcggtggcagctgcgaaacccagggagccgatgccacgtgacccaatgtggacttcttttaaacctttctaatgcccataacccagcctcagacccatggagcccacgagagactgcccgctgttcgggggcgccttttccgccatcctccccatgggggccattgacgtaagcgacctccgaccggtcccggacaatcaagaagttttctgccatcccgtgacggaccagagcctgatagtgaaacttctcgagctgcaggcccacgtacggggcgaagcggctgcgcggtaccactttgaggatgttggtggcgtgcagggggctagggctgtccatgtggagtctgttcagcctctcagtttggagaacctggccctgaggggccgctgtcaagaagcctgggtcctctctggcaagcagcagatagctaaggaaaaccagcaggtagcaaaggacgtgacacttcatcaggccttgctgaggctgccccagtaccagactgatctcttgcttaccttcaatcagcccccccctgacaacaggtcatctcttggccccgaaaatctgtcacctgcaccctggagcctgggtgactttgaacagctggtgaccagtctgacccttcacgatcctaacatctttggtccccagtaaaggcgctgaagcactgcatgatgttgctgagaacttggggactcggttctgtgagggggaaaagaggttgaaaagagggtttcctcttatttcttccctgtgcgtaaacataagacaatccctcttcagaataaacttgctttataatcaaaaaaaaaaaaaaaaaaa

SEQ ID NO: 2 - protein, 186 aa, Artificial Sequence
  MOG1 gene mutant
MEPTRDCPLFGGAFSAILPMGAIDVSDLRPVPDNQEVFCHPVTDQSLIVKLLELQAHVRGEAAARYHFEDVGGVQGARAVHVESVQPLSLENLALRGRCQEAWVLSGKQQIAKENQQVAKDVTLHQALLRLPQYQTDLLLTFNQPPPDNRSSLGPENLSPAPWSLGDFEQLVTSLTLHDPNIFGPQ